European Patent Specification EP 3 898 986 B1, published February 18, 2026. Title: LETTUCE PLANT RESISTANT TO DOWNY MILDEW AND RESISTANCE GENE. Applicant: ENZA ZADEN BEHEER B.V. The sequence listing filed with the application follows.

SEQUENCE LISTING (14 sequences)

SEQ ID NO: 1 - DNA, 2175 bp, Lactuca sativa
  SL7
atgcctgttgggatgatagaaagttggacaacattttacttatcaaataaggtcctcgatgacttacttcatgagttaccattgttgagagttctaagtttgagtcatcttagcatcaaggaggtacctgaaataataggcagtttgaaacacttgcggtatcttaatttatcacacactaccatcacacatttaccggaaaatatatgcaatctttacaacttacagacattgatcctttgtggctgttgttttataaccaagtttcccgacaacttcttaaagcttagaaatttacggcatttggacattagcgatactcccggtttgaagaagatgtcctcggggattggtgaattgaagaacctacacactctctccaaggtcattattggaggtgaaaatagactaaacgagcttaagaacttgcaaaatctccatgggaaaatttccgtttgggggttgggcgatgtgcaaaatgcaatggaggcacgtgaggcgaatttatcacaaaagaaacttagcgagttacagttggattggggttatggggattatgggttgaatgtttctcgaaagcaaacccatgataaggaggtccttaatgagctgaagcctgataacgatagtttgaaaaagcttgaaattttgtcatatggaggtacagagtttccaaattgggttgggaatccctcgtttcttatactaactcatgtgtccataaatttctgtgaagaatgtacatgtctaccaagtcttgggaagttaccatcacttaaggagctgtttattcttggcatgagcaaggtgaaagttattgatttggagttacttggaactggagttgcattcccatcacttgaaattctaagttttcgtcatatgtcagggtgggaggtatggtcaactgataatggtggggttgtagacacagcatttccatgtcttcaagaacttcatatcgaattttgtcctaatttagttcaagtctcacttgaagccctaccttcacttagagttttagaaataaaaggatgtggtcatggtgtgttgacaactctgcttcatgtagcttcttcagtcaccatgttggaaatagataatatttcagggcttactgatgaactgtggagaagtgttttcaagtatcttgggaaacttgaaaagttatacattagtgggtgtaatgaaataagatatttgtggcaatcagaagtagaggcaagtaagtctctagtgaatttaaggaatttgaatgtgagtgcttgttcaaatctggtgggtttaggagagaaagtggaggataactgtggaagcatccagacgtttattaggatgttgtctatagcacgttgtgagagtattgagcattgcagttgtcctaatagcattgagtttctgaatatccatgattgtgattcaattacatcagtgtctttcccaactggaggagggaagaagctcaagtcatttgcaattgaaggttgtcagaagtttttggaagaggaccttggaggagaaaagagtaggttgcttatcaaatcaagcatgcaaatgcttgaatctgtagatataaatggttgggtaaatctgaaatctatcattgaattaagttactgtattcacctcaccacattgatgataacaaagtgtccaaaaatggagtcgtttcccgaccatgagttacccaatctcacctctttaacaattctggtaatagcaaagtgtccaagtattgatgcctcctttcctcgtgggctttggcctcccaaattgagttaccttggaataggaggattgaagaagcccatctcagagtggggcccacagaatttcccaacctcactcgagaacttgatgttaaatggcggaatatatgatgatgtgaaaaactttgatcaattgtcgcatctttttccttcatctcttgcttctctttcgataatgggatttcagaaactggaatcagtttcaatgggactccaaaacctcacctttctccagcgtctctttgtttccaagtgcccgaagatgttacatctaccagaaaagttgtttccttcgcttttgtctttgagaatcgatggatgcccaaatttgaatgaaaggagcattagaagaagctcctattggcccctcatctcccttatcccagactccacttttgacgagtaa

SEQ ID NO: 2 - protein, 724 aa, Lactuca sativa
  SL7
MPVGMIESWTTFYLSNKVLDDLLHELPLLRVLSLSHLSIKEVPEIIGSLKHLRYLNLSHTTITHLPENICNLYNLQTLILCGCCFITKFPDNFLKLRNLRHLDISDTPGLKKMSSGIGELKNLHTLSKVIIGGENRLNELKNLQNLHGKISVWGLGDVQNAMEAREANLSQKKLSELQLDWGYGDYGLNVSRKQTHDKEVLNELKPDNDSLKKLEILSYGGTEFPNWVGNPSFLILTHVSINFCEECTCLPSLGKLPSLKELFILGMSKVKVIDLELLGTGVAFPSLEILSFRHMSGWEVWSTDNGGVVDTAFPCLQELHIEFCPNLVQVSLEALPSLRVLEIKGCGHGVLTTLLHVASSVTMLEIDNISGLTDELWRSVFKYLGKLEKLYISGCNEIRYLWQSEVEASKSLVNLRNLNVSACSNLVGLGEKVEDNCGSIQTFIRMLSIARCESIEHCSCPNSIEFLNIHDCDSITSVSFPTGGGKKLKSFAIEGCQKFLEEDLGGEKSRLLIKSSMQMLESVDINGWVNLKSIIELSYCIHLTTLMITKCPKMESFPDHELPNLTSLTILVIAKCPSIDASFPRGLWPPKLSYLGIGGLKKPISEWGPQNFPTSLENLMLNGGIYDDVKNFDQLSHLFPSSLASLSIMGFQKLESVSMGLQNLTFLQRLFVSKCPKMLHLPEKLFPSLLSLRIDGCPNLNERSIRRSSYWPLISLIPDSTFDE

SEQ ID NO: 3 - DNA, 2196 bp, Lactuca saligna
  SL7R
atgcctgttgggatgatagaaagttggacaagattttacttatcaaataaggtcctggatgacttacttcacgagttaccattgttgagagttctaagtttgagtcatcttaacatcacagaggtacctgaaataataggcaatttgaaacacttgcggtatcttaatttatctcacacgagtatcacacatttaccagaaaatgtctgcaatctttacaacttacaaacattgatcctttgtggctgtcgttttataaccaagtttcccaacaacttcttaaagcttagaaatttacggcatttggacattagcgatactcccggtttgaagaagatgtcctcggggattggtgaattgaagaacctacacactctctccaagatcattattggaggtgaaaatagactaaacgagcttaagaacttacaaaatctccatgggaaaatttccgtttgggggttgggcgatgtgcaaaatgcaatggaggcacgtgaggcgaatttatcacaaaagaaacttggcgagttacagttggattggggttatggggattatgagttgaatgtttctcgaaagcaaacccatgataaggaggtccttaatgagctgaagcctgataacgatagtttgaaaaagcttaaaattttgtcatatggaggtacagagtttccaaattgggttgggagtccctcgtttcttatgctaactcatgtgtccatatatttctgtgaagaatgtacatatctaccaagtcttgggaagttaccatcacttaaggagctgtttattcttggcatgagcaaggtgaaagttattgattgggagttacttggaactggagttgcattcccatcacttgaaattctaagttttggtcatatgtcagggtgggaggtatggtcaaccgagaatagtggggttgtagacacagcatttccatgtcttcaagaacttcatatcgaattttgtcctaatttagttcaagtctcacttgaagccctaccttcacttagagttttagaaataaaaggatgtggtcatggtgtgttgacaactctggttcatgtagcttcttcagtcaccatgttggaaataggtaatatttcagggcttaatgatgaactgtggagaagtgctttcaagtatcttgggaaacttgaaaagttatacattcgtgggtgtaatgaaataagatatttgtggcaatcagaagtagaggcaagtaagtctctagtgaatttaaggaatttggatgtgagtgattgttcaaatctggtgggtttaggagagaaagtggaggataactctggaagcatccagacgtttattaggatgttgtctatagcacgttgtgagactattgagcattgcagttgtcctaatagcattgagtttctgaatatccatgattgtgattcaattacatcagtgtctttcccaaaaggaggagggaagaagctcaagtcatttgccattgaaggttgtcagaagtttttggaagaggagctcggaggagaaaagagtaggttgcttatcaactcaaacatgaaaatgcttgaatctgtagatataaatggttgggtaaatctgaaatctatcattgaattgagttactgtattcacctcaccacattgatgataacaaagtgtccaaaaatggagtcttttcctgaccatgagttacccaatctcacctctttaacaattctgataatagcaaagtgtccaagtattgatgcctcctttcctcgtgggctttggcctcccaaattgagttaccttggaataggaggattgaagaagcccatctcagagtggggcccacagaatttcccaacctcactcgagcacttaatgttaaatggcggaatatatgatgatgtgaaaaactttgatcaattgtcgcatctttttccttcatctcttgcttctctttcgataacgggatttcagaaacttgaatcagtttcattgggactccaaaacctcacctttctccagcgtctctctgtttccaagtgcccaaagatgttacatctaccagaaaagttgcttccttcgcttttgtctttgagtatcgatagatgcccaaatttgaataaaaggagcattagaagaagctcctattggcccctcatctcccttatcccagactctaggtatgcccctctcaaagtttttgacttcttctag

SEQ ID NO: 4 - protein, 731 aa, Lactuca saligna
  SL7R
MPVGMIESWTRFYLSNKVLDDLLHELPLLRVLSLSHLNITEVPEIIGNLKHLRYLNLSHTSITHLPENVCNLYNLQTLILCGCRFITKFPNNFLKLRNLRHLDISDTPGLKKMSSGIGELKNLHTLSKIIIGGENRLNELKNLQNLHGKISVWGLGDVQNAMEAREANLSQKKLGELQLDWGYGDYELNVSRKQTHDKEVLNELKPDNDSLKKLKILSYGGTEFPNWVGSPSFLMLTHVSIYFCEECTYLPSLGKLPSLKELFILGMSKVKVIDWELLGTGVAFPSLEILSFGHMSGWEVWSTENSGVVDTAFPCLQELHIEFCPNLVQVSLEALPSLRVLEIKGCGHGVLTTLVHVASSVTMLEIGNISGLNDELWRSAFKYLGKLEKLYIRGCNEIRYLWQSEVEASKSLVNLRNLDVSDCSNLVGLGEKVEDNSGSIQTFIRMLSIARCETIEHCSCPNSIEFLNIHDCDSITSVSFPKGGGKKLKSFAIEGCQKFLEEELGGEKSRLLINSNMKMLESVDINGWVNLKSIIELSYCIHLTTLMITKCPKMESFPDHELPNLTSLTILIIAKCPSIDASFPRGLWPPKLSYLGIGGLKKPISEWGPQNFPTSLEHLMLNGGIYDDVKNFDQLSHLFPSSLASLSITGFQKLESVSLGLQNLTFLQRLSVSKCPKMLHLPEKLLPSLLSLSIDRCPNLNKRSIRRSSYWPLISLIPDSRYAPLKVFDFF

SEQ ID NO: 5 - DNA, 297 bp, Artificial Sequence
  VIGS construct 1A
ttcatgtagcttcttcagtcaccatgttggaaataggtaatatttcagggcttaatgatgaactgtggagaagtgctttcaagtatcttgggaaacttgaaaagttatacattcgtgggtgtaatgaaataagatatttgtggcaatcagaagtagaggcaagtaagtctctagtgaatttaaggaatttggatgtgagtgattgttcaaatctggtgggtttaggagagaaagtggaggataactctggaagcatccagacgtttattaggatgttgtctatagcacgttgtgaga

SEQ ID NO: 6 - DNA, 304 bp, Artificial Sequence
  VIGS construct 1B
tgagttaccttggaataggaggattgaagaagcccatctcagagtggggcccacagaatttcccaacctcactcgagcacttaatgttaaatggcggaatatatgatgatgtgaaaaactttgatcaattgtcgcatctttttccttcatctcttgcttctctttcgataacgggatttcagaaacttgaatcagtttcattgggactccaaaacctcacctttctccagcgtctctctgtttccaagtgcccaaagatgttacatctaccagaaaagttgcttccttcgcttttgtctttgag

SEQ ID NO: 7 - DNA, 183 bp, Artificial Sequence
  VIGS construct 2A
gtggagatcaagctggattataagaaggatttgtttgatgggaagaggaatattgtcacggcggaggagatagagagcgggataaggcggctgatggaggatgacgatgtaagagaaaagataaaagagatggggaaaaagagcaaagcgactgttaaagagggaggttcgtcttacgcttct

SEQ ID NO: 8 - DNA, 269 bp, Artificial Sequence
  VIGS construct 2B
cacattcttggaattagaaacacgcccaatcgagtcgttgtctaccgacagcaggataccgtctgtgtatccggtaggacctgtactgaacctagaagacggtgccggaacaccgccggaaagtgacgtcatcagctggttggacaatcaaccaccttcctcggttgttttcttgtgttttgggagtctgggatgttttgatgaagtccaagtgaaggagattgcatatgctttagagcgaagcgggcgttctttcttgtggtcactac

SEQ ID NO: 9 - DNA, 21 bp, Artificial Sequence
  QPCR primer
tccaagtattgatgcctcctt

SEQ ID NO: 10 - DNA, 21 bp, Artificial Sequence
  QPCR primer
cactctgagatgggcttcttc

SEQ ID NO: 11 - DNA, 20 bp, Artificial Sequence
  QPCR primer
gcgagaaattgtgcgtgata

SEQ ID NO: 12 - DNA, 20 bp, Artificial Sequence
  QPCR primer
actcggctgcagtcttcatt

SEQ ID NO: 13 - DNA, 24 bp, Artificial Sequence
  QPCR primer
cttcttagtgttcaatgctgttgg

SEQ ID NO: 14 - DNA, 24 bp, Artificial Sequence
  QPCR primer
gaagggtagatagtgaaaccgagc